European Patent Application EP 4 640 715 A1, published October 29, 2025. Title: MULTI-SPECIFIC POLYPEPTIDE COMPLEX TARGETING GPRC5D. Applicant: CHIMAGEN BIOSCIENCES, LTD. The sequence listing filed with the application follows.

SEQUENCE LISTING (112 sequences)

SEQ ID NO: 1 - protein, 5 aa, synthetic construct
  REGION 1..5: note = synthetic
SSVSF

SEQ ID NO: 2 - skipped

SEQ ID NO: 3 - protein, 9 aa, synthetic construct
  REGION 1..9: note = synthetic
QQWNSHPLT

SEQ ID NO: 4 - protein, 8 aa, synthetic construct
  REGION 1..8: note = synthetic
GYPFTNYW

SEQ ID NO: 5 - protein, 8 aa, synthetic construct
  REGION 1..8: note = synthetic
INPSNGRT

SEQ ID NO: 6 - protein, 6 aa, synthetic construct
  REGION 1..6: note = synthetic
ARGFAY

SEQ ID NO: 7 - protein, 10 aa, synthetic construct
  REGION 1..10: note = synthetic
SASSSVSFMH

SEQ ID NO: 8 - protein, 7 aa, synthetic construct
  REGION 1..7: note = synthetic
DTTKLAS

SEQ ID NO: 9 - protein, 5 aa, synthetic construct
  REGION 1..5: note = synthetic
NYWMH

SEQ ID NO: 10 - protein, 17 aa, synthetic construct
  REGION 1..17: note = synthetic
EINPSNGRTNYNEKFKS

SEQ ID NO: 11 - protein, 4 aa, synthetic construct
  REGION 1..4: note = synthetic
GFAY

SEQ ID NO: 12 - protein, 106 aa, synthetic construct
  REGION 1..106: note = synthetic
QIVLSQFPAIMSASPGEKVTMTCSASSSVSFMHWYQQKSGTSPKRWIYDTTKLASGVPARFTGSGSGTSYSLTISSMEAEDAATYYCQQWNSHPLTFGPGTKLELK

SEQ ID NO: 13 - protein, 113 aa, synthetic construct
  REGION 1..113: note = synthetic
QVQLQQPGAELVKPGTSVKLSCKASGYPFTNYWMHWVRQRPGQGLEWIGEINPSNGRTNYNEKFKSLATLTLDKSSSTAYMHLNSLTSEDSAVYYCARGFAYWGQGTLVTVSA

SEQ ID NO: 14 - protein, 106 aa, synthetic construct
  REGION 1..106: note = synthetic
EIVLTQSPGTLSLSPGERATLSCSASSSVSFMHWYQQKPGQAPRRWIYDTTKLASGIPDRFSGSGSGTDYTLTISRLEPEDFAVYYCQQWNSHPLTFGQGTTVEIK

SEQ ID NO: 15 - protein, 113 aa, synthetic construct
  REGION 1..113: note = synthetic
QVQLVQSGAEVKKPGSSVKVSCRASGYPFTNYWMHWVRQAPGQGLEWIGEINPSNGRTNYNEKFKSRATLTLDKLTSTAYMELSSLTSEDTALYYCARGFAYWGQGTLVTVSS

SEQ ID NO: 16 - protein, 106 aa, synthetic construct
  REGION 1..106: note = synthetic
EIVLTQSPATLSLSPGERATLSCSASSSVSFMHWYQQKPGQAPRRWIYDTTKLASGIPARFSGSGSGTDYTLTISSLEPEDFAVYYCQQWNSHPLTFGQGTKLEIK

SEQ ID NO: 17 - protein, 113 aa, synthetic construct
  REGION 1..113: note = synthetic
EVTLKESGPVLVKPTETLTLTCTASGYPFTNYWMHWVRQPPGKALEWIGEINPSNGRTNYNEKFKSRATLSLDKSKSQAVLTMTNMDPVDTATYYCARGFAYWGQGTLVTVSS

SEQ ID NO: 18 - protein, 106 aa, synthetic construct
  REGION 1..106: note = synthetic
EIVLTQSPATLSLSPGERATLSCSASSSVSFMHWYQQKPGQAPRRWIYDTTKLASGVPARFSGSGSGTDYTLTISSLEPEDFAVYYCQQWNSHPLTFGQGTKVEIK

SEQ ID NO: 19 - protein, 111 aa, synthetic construct
  REGION 1..111: note = synthetic
ELVQSGAEVKKPGSSVKVSCKASGYPFTNYWMHWVRQAPGQGLEWIGEINPSNGRTNYNEKFKSRATLTLDKSTSTAYMELSSLRSEDTAVYYCARGFAYWGQGTLVTVSS

SEQ ID NO: 20 - protein, 106 aa, synthetic construct
  REGION 1..106: note = synthetic
AIQLTQSPSSLSASVGDRVTITCSASSSVSFMHWYQQKPGKAPKRWIYDTTKLASGVPSRFSGSGSGTDYTFTISSLQPEDIATYYCQQWNSHPLTFGPGTKVDIK

SEQ ID NO: 21 - protein, 113 aa, synthetic construct
  REGION 1..113: note = synthetic
QVQLQESGPGLVKPSETLSLTCTASGYPFTNYWMHWVRQPPGKGLEWIGEINPSNGRTNYNEKFKSRATLSLDKSKNQASLNLDSVSAADTAIYYCARGFAYWGKGSTVTVSS

SEQ ID NO: 22 - protein, 236 aa, synthetic construct
  REGION 1..236: note = synthetic
QIVLSQFPAIMSASPGEKVTMTCSASSSVSFMHWYQKKSGTSPKRWIYDTTKLASGVPARFTGSGSGTSYSLTISSMEAEDAATYYCQQWNSHPLTFGCGTKLELKRTVAAEVQLVESGGGLVQPGGSLRLSCAASGFTFSTYAMNWVRQAPGKGLEWVGRIRSKYNNYATYYADSVKGRFTISRDDSKNSLYLQMNSLRAEDTAVYYCVRHGNFGNSYVSWFAYWGQGTLVTVSS

SEQ ID NO: 23 - protein, 227 aa, synthetic construct
  REGION 1..227: note = synthetic
QAVVTQEPSLTVSPGGTVTLTCRSSTGAVTTSNYANWVQQKPGQAPRGLIGGTNKRAPWTPARFSGSLLGGKAALTLSGAQAEDEADYYCALWYSNLWVFGGGTKLTVLRTVAAQVQLQQPGAELVKPGTSVKLSCKASGYPFTNYWMHWVRDRPGQCLEWIGEINPSNGRTNYNEKFKSLATLTLDKSSSTAYMHLNSLTSEDSAVYYCARGFAYWGQGTLVTVSS

SEQ ID NO: 24 - protein, 224 aa, synthetic construct
  REGION 1..224: note = synthetic
DKTHTCPPCPAPPVAGPSVFLFPPKPKDTLMISRTPEVTCVVVDVSQEDPEVKFNWYVDGVEVHNAKTKPREEQFNSTYRVVSVLTVLHQDWLNGKEYKCKVSNKGLPSSIEKTISKAKGQPREPQVYTLPPSRDELTKNQVSLSCAVKGFYPSDIAVEWESNGQPENNYKTTPPVLDSDGSFFLVSKLTVDKSRWQQGNVFSCSVMHEALHNRFTQKSLSLSP

SEQ ID NO: 25 - protein, 237 aa, synthetic construct
  REGION 1..237: note = synthetic
DIQMTQSPSSLSASVGDRVTITCRASQDVNTAVAWYQDKPGKAPKLLIYSASFLYSGVPSRFSGSRSGTDFTLTISSLQPEDFATYYCQQAYTTPPTFGCGTKVEIKRTVAAEVQLVESGGGLVQPGGSLRLSCAASGFTFSTYAMNWVRDAPGKGLEWVGRIRSKYNNYATYYADSVKGRFTISRDDSKNSLYLQMNSLRAEDTAVYYCVRHGNFGNSYVSWFAYWGQGTLVTVSS

SEQ ID NO: 26 - protein, 234 aa, synthetic construct
  REGION 1..234: note = synthetic
QAVVTQEPSLTVSPGGTVTLTCRSSTGAVTTSNYANWVQKKPGQAPRGLIGGTNKRAPWTPARFSGSLLGGKAALTLSGAQAEDEADYYCALWYSNLWVFGGGTKLTVLRTVAAEVQLVESGGGLVQPGGSLRLSCAASGFNIKDTYIHWVRKAPGKCLEWVARIYPTNGYTRYADSVKGRFTISADTSKNTAYLQMNSLRAEDTAVYYCSRWGGDGFYAMDYWGQGTLVTVSS

SEQ ID NO: 27 - protein, 216 aa, synthetic construct
  REGION 1..216: note = synthetic
QVQLQQPGAELVKPGTSVKLSCKASGYPFTNYWMHWVRQRPGQGLEWIGEINPSNGRTNYNEKFKSLATLTLDKSSSTAYMHLNSLTSEDSAVYYCARGFAYWGQGTLVTVSSASTKGPSVFPLAPSSKSTSGGTAALGCLVKDYFPEPVTVSWNSGALTSGVHTFPAVLQSSGLYSLSSVVTVPSSSLGTQTYICNVNHKPSNTKVDKKVEPKSC

SEQ ID NO: 28 - protein, 213 aa, synthetic construct
  REGION 1..213: note = synthetic
QIVLSQFPAIMSASPGEKVTMTCSASSSVSFMHWYQQKSGTSPKRWIYDTTKLASGVPARFTGSGSGTSYSLTISSMEAEDAATYYCQQWNSHPLTFGPGTKLELKRTVAAPSVFIFPPSDEQLKSGTASVVCLLNNFYPREAKVQWKVDNALQSGNSQESVTEQDSKDSTYSLSSTLTLSKADYEKHKVYACEVTHQGLSSPVTKSFNRGEC

SEQ ID NO: 29 - protein, 236 aa, synthetic construct; identical to SEQ ID NO: 22
  REGION 1..236: note = synthetic

SEQ ID NO: 30 - protein, 227 aa, synthetic construct; identical to SEQ ID NO: 23
  REGION 1..227: note = synthetic

SEQ ID NO: 31 - protein, 216 aa, synthetic construct; identical to SEQ ID NO: 27
  REGION 1..216: note = synthetic

SEQ ID NO: 32 - protein, 213 aa, synthetic construct; identical to SEQ ID NO: 28
  REGION 1..213: note = synthetic

SEQ ID NO: 33 - protein, 224 aa, synthetic construct
  REGION 1..224: note = synthetic
QIVLSQFPAIMSASPGEKVTMTCSASSSVSFMHWYQKKSGTSPKRWIYDTTKLASGVPARFTGSGSGTSYSLTISSMEAEDAATYYCQQWNSHPLTFGCGTKLELKRTVAAQVQLQQPGAELVKPGTSVKLSCKASGYPFTNYWMHWVRQRPGQGLEWIGEINPSNGRTNYNEKFKSLATLTLDKSSSTAYMHLNSLTSEDSAVYYCARGFAYWGQGTLVTVSS

SEQ ID NO: 34 - protein, 224 aa, synthetic construct
  REGION 1..224: note = synthetic
QIVLSQFPAIMSASPGEKVTMTCSASSSVSFMHWYQQKSGTSPKRWIYDTTKLASGVPARFTGSGSGTSYSLTISSMEAEDAATYYCQQWNSHPLTFGPGTKLELKRTVAAQVQLQQPGAELVKPGTSVKLSCKASGYPFTNYWMHWVRDRPGQCLEWIGEINPSNGRTNYNEKFKSLATLTLDKSSSTAYMHLNSLTSEDSAVYYCARGFAYWGQGTLVTVSS

SEQ ID NO: 35 - protein, 228 aa, synthetic construct
  REGION 1..228: note = synthetic
EVQLVESGGGLVQPGGSLRLSCAASGFTFSTYAMNWVRQAPGKGLEWVGRIRSKYNNYATYYADSVKGRFTISRDDSKNSLYLQMNSLRAEDTAVYYCVRHGNFGNSYVSWFAYWGQGTLVTVSSASTKGPSVFPLAPSSKSTSGGTAALGCLVKDYFPEPVTVSWNSGALTSGVHTFPAVLQSSGLYSLSSVVTVPSSSLGTQTYICNVNHKPSNTKVDKKVEPKSC

SEQ ID NO: 36 - protein, 216 aa, synthetic construct
  REGION 1..216: note = synthetic
QAVVTQEPSLTVSPGGTVTLTCRSSTGAVTTSNYANWVQQKPGQAPRGLIGGTNKRAPWTPARFSGSLLGGKAALTLSGAQAEDEADYYCALWYSNLWVFGGGTKLTVLRTVAAPSVFIFPPSDEQLKSGTASVVCLLNNFYPREAKVQWKVDNALQSGNSQESVTEQDSKDSTYSLSSTLTLSKADYEKHKVYACEVTHQGLSSPVTKSFNRGEC

SEQ ID NO: 37 - protein, 216 aa, synthetic construct
  REGION 1..216: note = synthetic
QAVVTQEPSLTVSPGGTVTLTCRSSTGAVTTSNYANWVQKKPGQAPRGLIGGTNKRAPWTPARFSGSLLGGKAALTLSGAQAEDEADYYCALWYSNLWVFGGGTKLTVLRTVAAPSVDIFPPSDEQLKSGTASVVCLLNNFYPREAKVQWKVDNALQSGNSCESVTEQDSKDSTYSLSSTLTLSKADYEKHKVYACEVTHQGLSSPVTKSFNRGES

SEQ ID NO: 38 - protein, 228 aa, synthetic construct
  REGION 1..228: note = synthetic
EVQLVESGGGLVQPGGSLRLSCAASGFTFSTYAMNWVRDAPGKGLEWVGRIRSKYNNYATYYADSVKGRFTISRDDSKNSLYLQMNSLRAEDTAVYYCVRHGNFGNSYVSWFAYWGQGTLVTVSSASTKGPSVFPLAPSSKSTSGGTAKLGCLVKDYFPEPVTVSWNSGALTSGVHTFPACLQSSGLYSLSSVVTVPSSSLGTQTYICNVNHKPSNTKVDKKVEPKSS

SEQ ID NO: 39 - protein, 216 aa, synthetic construct; identical to SEQ ID NO: 27
  REGION 1..216: note = synthetic

SEQ ID NO: 40 - protein, 213 aa, synthetic construct; identical to SEQ ID NO: 28
  REGION 1..213: note = synthetic

SEQ ID NO: 41 - protein, 443 aa, synthetic construct
  REGION 1..443: note = synthetic
QVQLQQPGAELVKPGTSVKLSCKASGYPFTNYWMHWVRQRPGQGLEWIGEINPSNGRTNYNEKFKSLATLTLDKSSSTAYMHLNSLTSEDSAVYYCARGFAYWGQGTLVTVSSASTKGPSVFPLAPSSKSTSGGTAALGCLVKDYFPEPVTVSWNSGALTSGVHTFPAVLQSSGLYSLSSVVTVPSSSLGTQTYICNVNHKPSNTKVDKKVEPKSCDGGGGSGGGGSQAVVTQEPSLTVSPGGTVTLTCRSSTGAVTTSNYANWVQKKPGQAPRGLIGGTNKRAPWTPARFSGSLLGGKAALTLSGAQAEDEADYYCALWYSNLWVFGGGTKLTVLRTVAAPSVDIFPPSDEQLKSGTASVVCLLNNFYPREAKVQWKVDNALQSGNSCESVTEQDSKDSTYSLSSTLTLSKADYEKHKVYACEVTHQGLSSPVTKSFNRGES

SEQ ID NO: 42 - protein, 228 aa, synthetic construct; identical to SEQ ID NO: 38
  REGION 1..228: note = synthetic

SEQ ID NO: 43 - protein, 216 aa, synthetic construct; identical to SEQ ID NO: 27
  REGION 1..216: note = synthetic

SEQ ID NO: 44 - protein, 213 aa, synthetic construct; identical to SEQ ID NO: 28
  REGION 1..213: note = synthetic

SEQ ID NO: 45 - protein, 443 aa, synthetic construct
  REGION 1..443: note = synthetic
QVQLVQSGAEVKKPGSSVKVSCRASGYPFTNYWMHWVRQAPGQGLEWIGEINPSNGRTNYNEKFKSRATLTLDKLTSTAYMELSSLTSEDTALYYCARGFAYWGQGTLVTVSSASTKGPSVFPLAPSSKSTSGGTAALGCLVKDYFPEPVTVSWNSGALTSGVHTFPAVLQSSGLYSLSSVVTVPSSSLGTQTYICNVNHKPSNTKVDKKVEPKSCDGGGGSGGGGSQAVVTQEPSLTVSPGGTVTLTCRSSTGAVTTSNYANWVQQKPGQAPRGLIGGTNKRAPWTPARFSGSLLGGKAALTLSGAQAEDEADYYCALWYSNLWVFGGGTKLTVLRTVAAPSVDIFPPSDEQLKSGTASVVCLLNNFYPREAKVQWKVDNALQSGNSCESVTEQDSKDSTYSLSSTLTLSKADYEKHKVYACEVTHQGLSSPVTKSFNRGES

SEQ ID NO: 46 - protein, 228 aa, synthetic construct
  REGION 1..228: note = synthetic
EVQLVESGGGLVQPGGSLRLSCAASGFTFSTYAMNWVRQAPGKGLEWVGRIRSKYNNYATYYADSVKGRFTISRDDSKNSLYLQMNSLRAEDTAVYYCVRHGNFGTSYVSWFAYWGQGTLVTVSSASTKGPSVFPLAPSSKSTSGGTAKLGCLVKDYFPEPVTVSWNSGALTSGVHTFPACLQSSGLYSLSSVVTVPSSSLGTQTYICNVNHKPSNTKVDKKVEPKSS

SEQ ID NO: 47 - protein, 216 aa, synthetic construct
  REGION 1..216: note = synthetic
QVQLVQSGAEVKKPGSSVKVSCRASGYPFTNYWMHWVRQAPGQGLEWIGEINPSNGRTNYNEKFKSRATLTLDKLTSTAYMELSSLTSEDTALYYCARGFAYWGQGTLVTVSSASTKGPSVFPLAPSSKSTSGGTAALGCLVKDYFPEPVTVSWNSGALTSGVHTFPAVLQSSGLYSLSSVVTVPSSSLGTQTYICNVNHKPSNTKVDKKVEPKSC

SEQ ID NO: 48 - protein, 213 aa, synthetic construct
  REGION 1..213: note = synthetic
EIVLTQSPGTLSLSPGERATLSCSASSSVSFMHWYQQKPGQAPRRWIYDTTKLASGIPDRFSGSGSGTDYTLTISRLEPEDFAVYYCQQWNSHPLTFGQGTTVEIKRTVAAPSVFIFPPSDEQLKSGTASVVCLLNNFYPREAKVQWKVDNALQSGNSQESVTEQDSKDSTYSLSSTLTLSKADYEKHKVYACEVTHQGLSSPVTKSFNRGEC

SEQ ID NO: 49 - protein, 5 aa, synthetic construct
  REGION 1..5: note = synthetic
TYAMN

SEQ ID NO: 50 - protein, 19 aa, synthetic construct
  REGION 1..19: note = synthetic
RIRSKYNNYATYYADSVKG

SEQ ID NO: 51 - protein, 14 aa, synthetic construct
  REGION 1..14: note = synthetic
HGNFGTSYVSWFAY

SEQ ID NO: 52 - protein, 14 aa, synthetic construct
  REGION 1..14: note = synthetic
RSSTGAVTTSNYAN

SEQ ID NO: 53 - protein, 7 aa, synthetic construct
  REGION 1..7: note = synthetic
GTNKRAP

SEQ ID NO: 54 - protein, 9 aa, synthetic construct
  REGION 1..9: note = synthetic
ALWYSNLWV

SEQ ID NO: 55 - protein, 125 aa, synthetic construct
  REGION 1..125: note = synthetic
EVQLVESGGGLVQPGGSLRLSCAASGFTFSTYAMNWVRQAPGKGLEWVGRIRSKYNNYATYYADSVKGRFTISRDDSKNSLYLQMNSLRAEDTAVYYCVRHGNFGTSYVSWFAYWGQGTLVTVSS

SEQ ID NO: 56 - protein, 109 aa, synthetic construct
  REGION 1..109: note = synthetic
QAVVTQEPSLTVSPGGTVTLTCRSSTGAVTTSNYANWVQQKPGQAPRGLIGGTNKRAPWTPARFSGSLLGGKAALTLSGAQAEDEADYYCALWYSNLWVFGGGTKLTVL

SEQ ID NO: 57 - protein, 8 aa, synthetic construct
  REGION 1..8: note = synthetic
GFNIKDTY

SEQ ID NO: 58 - protein, 8 aa, synthetic construct
  REGION 1..8: note = synthetic
IYPTNGYT

SEQ ID NO: 59 - protein, 13 aa, synthetic construct
  REGION 1..13: note = synthetic
SRWGGDGFYAMDY

SEQ ID NO: 60 - protein, 6 aa, synthetic construct
  REGION 1..6: note = synthetic
QDVNTA

SEQ ID NO: 61 - skipped

SEQ ID NO: 62 - protein, 9 aa, synthetic construct
  REGION 1..9: note = synthetic
QQHYTTPPT

SEQ ID NO: 63 - protein, 120 aa, synthetic construct [sequence omitted]

SEQ ID NO: 64 - protein, 107 aa, synthetic construct
  REGION 1..107: note = synthetic
DIQMTQSPSSLSASVGDRVTITCRASQDVNTAVAWYQQKPGKAPKLLIYSASFLYSGVPSRFSGSRSGTDFTLTISSLQPEDFATYYCQQAYTTPPTFGQGTKVEIK

SEQ ID NO: 65 - protein, 224 aa, synthetic construct; identical to SEQ ID NO: 24
  REGION 1..224: note = synthetic

SEQ ID NO: 66 - protein, 231 aa, synthetic construct
  REGION 1..231: note = synthetic
ASEPKSSDKTHTCPPCPAPPVAGPSVFLFPPKPKDTLMISRTPEVTCVVVDVSQEDPEVKFNWYVDGVEVHNAKTKPREEQFNSTYRVVSVLTVLHQDWLNGKEYKCKVSNKGLPSSIEKTISKAKGQPREPQVYTLPPSRDELTKNQVSLWCLVKGFYPSDIAVEWESNGQPENNYKTTPPVLDSDGSFFLYSKLTVDKSRWQQGNVFSCSVMHEALHNHYTQKSLSLSP

SEQ ID NO: 67 - protein, 225 aa, synthetic construct
  REGION 1..225: note = synthetic
DKTHTCPPCPAPELLAGPDVFLFPPKPKDTLMISRTPEVTCVVVDVSHEDPEVKFNWYVDGVEVHNAKTKPREEQYNSTYRVVSVLTVLHQDWLNGKEYKCKVSNKALPLPEEKTISKAKGQPREPQVYTLPPSRDELTKNQVSLWCLVKGFYPSDIAVEWESNGQPENNYKTTPPVLDSDGSFFLYSKLTVDKSRWQQGNVFSCSVMHEALHNHYTQKSLSLSP

SEQ ID NO: 68-69 - skipped (2 entries)

SEQ ID NO: 70 - protein, 214 aa, synthetic construct
  REGION 1..214: note = synthetic
DIQMTQSPSSLSASVGDRVTITCKASQNVATHVGWYQQKPGKAPKRLIYSASYRYSGVPSRFSGSGSGTEFTLTISNLQPEDFATYYCQQYNRYPYTFGQGTKLEIKRTVAAPSVFIFPPSDEQLKSGTASVVCLLNNFYPREAKVQWKVDNALQSGNSCESVTEQDSKDSTYSLDSTLTLSKADYEKHKVYACEVTHQGLSSPVTKSFNRGES

SEQ ID NO: 71 - protein, 442 aa, synthetic construct
  REGION 1..442: note = synthetic
QVQLVQSGAEVKKPGASVKVSCKASGYSFTGYTMNWVRQAPGQGLEWMGLINPYNSDTNYAQKLQGRVTMTTDTSTSTAYMELRSLRSDDTAVYYCARVALRVALDYWGQGTLVTVSSASTKGPSVFPLAPSSKSTSGGTAALGCLVKDYFPEPVTVSWNSGALTSGVHTFPACLQSSGLYSLKSVVTVPSSSLGTQTYICNVNHKPSNTKVDKKVESKYGPPCPPCPAPPVAGPSVFLFPPKPKDTLMISRTPEVTCVVVDVSQEDPEVKFNWYVDGVEVHNAKTKPREEQFNSTYRVVSVLTVLHQDWLNGKEYKCKVSNKGLPSSIEKTISKAKGQPREPQVYTLPPSRDELTKNQVSLWCLVKGFYPSDIAVEWESNGQPENNYKTTPPVLDSDGSFFLYSKLTVDKSRWQQGNVFSCSVMHEALHNHYTQKSLSLSP

SEQ ID NO: 72 - protein, 449 aa, synthetic construct
  REGION 1..449: note = synthetic
EVQLVESGGGLVQPGGSLRLSCAASGFTFNTYAMNWVRQAPGKGLEWVARIRSKYNNYATYYAASVKGRFTISRDDSKNSLYLQMNSLKTEDTAVYYCARHGNFGNSYVSWFAYWGQGTLVTVSSASTKGPSVFPLAPCSRSTSESTAALGCLVKDYFPEPVTVSWNSGALTSGVHTFPAVLQSSGLYSLSSVVTVPSSSLGTKTYTCNVDHKPSNTKVDKRVESKYGPPCPPCPAPPVAGPSVFLFPPKPKDTLMISRTPEVTCVVVDVSQEDPEVKFNWYVDGVEVHNAKTKPREEQFNSTYRVVSVLTVLHQDWLNGKEYKCKVSNKGLPSSIEKTISKAKGQPREPQVYTLPPSRDELTKNQVSLSCAVKGFYPSDIAVEWESNGQPENNYKTTPPVLDSDGSFFLVSKLTVDKSRWQQGNVFSCSVMHEALHNRFTQKSLSLSP

SEQ ID NO: 73 - protein, 215 aa, synthetic construct
  REGION 1..215: note = synthetic
QTVVTQEPSLTVSPGGTVTLTCRSSTGAVTTSNYANWVQQKPGQAPRGLIGGTNKRAPGTPARFSGSLLGGKAALTLSGVQPEDEAEYYCALWYSNLWVFGGGTKLTVLGQPKAAPSVTLFPPSSEELQANKATLVCLISDFYPGAVTVAWKADSSPVKAGVETTTPSKQSNNKYAASSYLSLTPEQWKSHRSYSCQVTHEGSTVEKTVAPTECS

SEQ ID NO: 74 - protein, 5 aa, synthetic construct
  REGION 1..5: note = synthetic
RTVAA

SEQ ID NO: 75 - protein, 458 aa, synthetic construct
  REGION 1..458: note = synthetic
QAVVTQEPSLTVSPGGTVTLTCRSSTGAVTTSNYANWVQQKPGQAPRGLIGGTNKRAPWTPARFSGSLLGGKAALTLSGAQAEDEADYYCALWYSNLWVFGGGTKLTVLRTVAAQVQLQQPGAELVKPGTSVKLSCKASGYPFTNYWMHWVRDRPGQCLEWIGEINPSNGRTNYNEKFKSLATLTLDKSSSTAYMHLNSLTSEDSAVYYCARGFAYWGQGTLVTVSSASEPKSSDKTHTCPPCPAPPVAGPSVFLFPPKPKDTLMISRTPEVTCVVVDVSQEDPEVKFNWYVDGVEVHNAKTKPREEQFNSTYRVVSVLTVLHQDWLNGKEYKCKVSNKGLPSSIEKTISKAKGQPREPQVYTLPPSRDELTKNQVSLWCLVKGFYPSDIAVEWESNGQPENNYKTTPPVLDSDGSFFLYSKLTVDKSRWQQGNVFSCSVMHEALHNHYTQKSLSLSP

SEQ ID NO: 76 - protein, 465 aa, synthetic construct
  REGION 1..465: note = synthetic
QAVVTQEPSLTVSPGGTVTLTCRSSTGAVTTSNYANWVQKKPGQAPRGLIGGTNKRAPWTPARFSGSLLGGKAALTLSGAQAEDEADYYCALWYSNLWVFGGGTKLTVLRTVAAEVQLVESGGGLVQPGGSLRLSCAASGFNIKDTYIHWVRKAPGKCLEWVARIYPTNGYTRYADSVKGRFTISADTSKNTAYLQMNSLRAEDTAVYYCSRWGGDGFYAMDYWGQGTLVTVSSASEPKSSDKTHTCPPCPAPPVAGPSVFLFPPKPKDTLMISRTPEVTCVVVDVSQEDPEVKFNWYVDGVEVHNAKTKPREEQFNSTYRVVSVLTVLHQDWLNGKEYKCKVSNKGLPSSIEKTISKAKGQPREPQVYTLPPSRDELTKNQVSLWCLVKGFYPSDIAVEWESNGQPENNYKTTPPVLDSDGSFFLYSKLTVDKSRWQQGNVFSCSVMHEALHNHYTQKSLSLSP

SEQ ID NO: 77 - protein, 440 aa, synthetic construct
  REGION 1..440: note = synthetic
QVQLQQPGAELVKPGTSVKLSCKASGYPFTNYWMHWVRQRPGQGLEWIGEINPSNGRTNYNEKFKSLATLTLDKSSSTAYMHLNSLTSEDSAVYYCARGFAYWGQGTLVTVSSASTKGPSVFPLAPSSKSTSGGTAALGCLVKDYFPEPVTVSWNSGALTSGVHTFPAVLQSSGLYSLSSVVTVPSSSLGTQTYICNVNHKPSNTKVDKKVEPKSCDKTHTCPPCPAPPVAGPSVFLFPPKPKDTLMISRTPEVTCVVVDVSQEDPEVKFNWYVDGVEVHNAKTKPREEQFNSTYRVVSVLTVLHQDWLNGKEYKCKVSNKGLPSSIEKTISKAKGQPREPQVYTLPPSRDELTKNQVSLSCAVKGFYPSDIAVEWESNGQPENNYKTTPPVLDSDGSFFLVSKLTVDKSRWQQGNVFSCSVMHEALHNRFTQKSLSLSP

SEQ ID NO: 78 - protein, 458 aa, synthetic construct; identical to SEQ ID NO: 75
  REGION 1..458: note = synthetic

SEQ ID NO: 79 - protein, 440 aa, synthetic construct; identical to SEQ ID NO: 77
  REGION 1..440: note = synthetic

SEQ ID NO: 80 - protein, 455 aa, synthetic construct
  REGION 1..455: note = synthetic
QIVLSQFPAIMSASPGEKVTMTCSASSSVSFMHWYQQKSGTSPKRWIYDTTKLASGVPARFTGSGSGTSYSLTISSMEAEDAATYYCQQWNSHPLTFGPGTKLELKRTVAAQVQLQQPGAELVKPGTSVKLSCKASGYPFTNYWMHWVRDRPGQCLEWIGEINPSNGRTNYNEKFKSLATLTLDKSSSTAYMHLNSLTSEDSAVYYCARGFAYWGQGTLVTVSSASEPKSSDKTHTCPPCPAPPVAGPSVFLFPPKPKDTLMISRTPEVTCVVVDVSQEDPEVKFNWYVDGVEVHNAKTKPREEQFNSTYRVVSVLTVLHQDWLNGKEYKCKVSNKGLPSSIEKTISKAKGQPREPQVYTLPPSRDELTKNQVSLWCLVKGFYPSDIAVEWESNGQPENNYKTTPPVLDSDGSFFLYSKLTVDKSRWQQGNVFSCSVMHEALHNHYTQKSLSLSP

SEQ ID NO: 81 - protein, 452 aa, synthetic construct
  REGION 1..452: note = synthetic
EVQLVESGGGLVQPGGSLRLSCAASGFTFSTYAMNWVRQAPGKGLEWVGRIRSKYNNYATYYADSVKGRFTISRDDSKNSLYLQMNSLRAEDTAVYYCVRHGNFGNSYVSWFAYWGQGTLVTVSSASTKGPSVFPLAPSSKSTSGGTAALGCLVKDYFPEPVTVSWNSGALTSGVHTFPAVLQSSGLYSLSSVVTVPSSSLGTQTYICNVNHKPSNTKVDKKVEPKSCDKTHTCPPCPAPPVAGPSVFLFPPKPKDTLMISRTPEVTCVVVDVSQEDPEVKFNWYVDGVEVHNAKTKPREEQFNSTYRVVSVLTVLHQDWLNGKEYKCKVSNKGLPSSIEKTISKAKGQPREPQVYTLPPSRDELTKNQVSLSCAVKGFYPSDIAVEWESNGQPENNYKTTPPVLDSDGSFFLVSKLTVDKSRWQQGNVFSCSVMHEALHNRFTQKSLSLSP

SEQ ID NO: 82 - protein, 453 aa, synthetic construct
  REGION 1..453: note = synthetic
EVQLVESGGGLVQPGGSLRLSCAASGFTFSTYAMNWVRDAPGKGLEWVGRIRSKYNNYATYYADSVKGRFTISRDDSKNSLYLQMNSLRAEDTAVYYCVRHGNFGNSYVSWFAYWGQGTLVTVSSASTKGPSVFPLAPSSKSTSGGTAKLGCLVKDYFPEPVTVSWNSGALTSGVHTFPACLQSSGLYSLSSVVTVPSSSLGTQTYICNVNHKPSNTKVDKKVEPKSSDKTHTCPPCPAPELLAGPDVFLFPPKPKDTLMISRTPEVTCVVVDVSHEDPEVKFNWYVDGVEVHNAKTKPREEQYNSTYRVVSVLTVLHQDWLNGKEYKCKVSNKALPLPEEKTISKAKGQPREPQVYTLPPSRDELTKNQVSLWCLVKGFYPSDIAVEWESNGQPENNYKTTPPVLDSDGSFFLYSKLTVDKSRWQQGNVFSCSVMHEALHNHYTQKSLSLSP

SEQ ID NO: 83 - protein, 440 aa, synthetic construct; identical to SEQ ID NO: 77
  REGION 1..440: note = synthetic

SEQ ID NO: 84 - protein, 453 aa, synthetic construct; identical to SEQ ID NO: 82
  REGION 1..453: note = synthetic

SEQ ID NO: 85 - protein, 440 aa, synthetic construct; identical to SEQ ID NO: 77
  REGION 1..440: note = synthetic

SEQ ID NO: 86 - protein, 453 aa, synthetic construct
  REGION 1..453: note = synthetic
EVQLVESGGGLVQPGGSLRLSCAASGFTFSTYAMNWVRQAPGKGLEWVGRIRSKYNNYATYYADSVKGRFTISRDDSKNSLYLQMNSLRAEDTAVYYCVRHGNFGTSYVSWFAYWGQGTLVTVSSASTKGPSVFPLAPSSKSTSGGTAKLGCLVKDYFPEPVTVSWNSGALTSGVHTFPACLQSSGLYSLSSVVTVPSSSLGTQTYICNVNHKPSNTKVDKKVEPKSSDKTHTCPPCPAPELLAGPDVFLFPPKPKDTLMISRTPEVTCVVVDVSHEDPEVKFNWYVDGVEVHNAKTKPREEQYNSTYRVVSVLTVLHQDWLNGKEYKCKVSNKALPLPEEKTISKAKGQPREPQVYTLPPSRDELTKNQVSLWCLVKGFYPSDIAVEWESNGQPENNYKTTPPVLDSDGSFFLYSKLTVDKSRWQQGNVFSCSVMHEALHNHYTQKSLSLSP

SEQ ID NO: 87 - protein, 440 aa, synthetic construct
  REGION 1..440: note = synthetic
QVQLVQSGAEVKKPGSSVKVSCRASGYPFTNYWMHWVRQAPGQGLEWIGEINPSNGRTNYNEKFKSRATLTLDKLTSTAYMELSSLTSEDTALYYCARGFAYWGQGTLVTVSSASTKGPSVFPLAPSSKSTSGGTAALGCLVKDYFPEPVTVSWNSGALTSGVHTFPAVLQSSGLYSLSSVVTVPSSSLGTQTYICNVNHKPSNTKVDKKVEPKSCDKTHTCPPCPAPPVAGPSVFLFPPKPKDTLMISRTPEVTCVVVDVSQEDPEVKFNWYVDGVEVHNAKTKPREEQFNSTYRVVSVLTVLHQDWLNGKEYKCKVSNKGLPSSIEKTISKAKGQPREPQVYTLPPSRDELTKNQVSLSCAVKGFYPSDIAVEWESNGQPENNYKTTPPVLDSDGSFFLVSKLTVDKSRWQQGNVFSCSVMHEALHNRFTQKSLSLSP

SEQ ID NO: 88 - protein, 445 aa, synthetic construct
  REGION 1..445: note = synthetic
QVQLVQSGAEVKKPGASVKVSCKASGYSFTGYTMNWVRQAPGQGLEWMGLINPYNSDTNYAQKLQGRVTMTTDTSTSTAYMELRSLRSDDTAVYYCARVALRVALDYWGQGTLVTVSSASTKGPSVFPLAPCSRSTSESTAALGCLVKDYFPEPVTVSWNSGALTSGVHTFPAVLQSSGLYSLSSVVTVPSSSLGTKTYTCNVDHKPSNTKVDKRVESKYGPPCPPCPAPEFLGGPSVFLFPPKPKDTLMISRTPEVTCVVVDVSQEDPEVQFNWYVDGVEVHNAKTKPREEQFNSTYRVVSVLTVLHQDWLNGKEYKCKVSNKGLPSSIEKTISKAKGQPREPQVYTLPPSQEEMTKNQVSLTCLVKGFYPSDIAVEWESNGQPENNYKTTPPVLDSDGSFFLYSRLTVDKSRWQEGNVFSCSVMHEALHNHYTQKSLSLSLGK

SEQ ID NO: 89 - protein, 214 aa, synthetic construct
  REGION 1..214: note = synthetic
DIQMTQSPSSLSASVGDRVTITCKASQNVATHVGWYQQKPGKAPKRLIYSASYRYSGVPSRFSGSGSGTEFTLTISNLQPEDFATYYCQQYNRYPYTFGQGTKLEIKRTVAAPSVFIFPPSDEQLKSGTASVVCLLNNFYPREAKVQWKVDNALQSGNSQESVTEQDSKDSTYSLSSTLTLSKADYEKHKVYACEVTHQGLSSPVTKSFNRGEC

SEQ ID NO: 90 - protein, 441 aa, synthetic construct
  REGION 1..441: note = synthetic
QVQLQQPGAELVKPGTSVKLSCKASGYPFTNYWMHWVRQRPGQGLEWIGEINPSNGRTNYNEKFKSLATLTLDKSSSTAYMHLNSLTSEDSAVYYCARGFAYWGQGTLVTVSSASTKGPSVFPLAPSSKSTSGGTAALGCLVKDYFPEPVTVSWNSGALTSGVHTFPAVLQSSGLYSLSSVVTVPSSSLGTQTYICNVNHKPSNTKVDKKVEPKSCDKTHTCPPCPAPELLGGPSVFLFPPKPKDTLMISRTPEVTCVVVDVSHEDPEVKFNWYVDGVEVHNAKTKPREEQYNSTYRVVSVLTVLHQDWLNGKEYKCKVSNKALPAPIEKTISKAKGQPREPQVYTLPPSRDELTKNQVSLTCLVKGFYPSDIAVEWESNGQPENNYKTTPPVLDSDGSFFLYSKLTVDKSRWQQGNVFSCSVMHEALHNHYTQKSLSLSP

SEQ ID NO: 91 - protein, 213 aa, synthetic construct; identical to SEQ ID NO: 28
  REGION 1..213: note = synthetic

SEQ ID NO: 92 - protein, 8 aa, synthetic construct
  REGION 1..8: note = synthetic
GFTFSTYA

SEQ ID NO: 93 - protein, 10 aa, synthetic construct
  REGION 1..10: note = synthetic
IRSKYNNYAT

SEQ ID NO: 94 - protein, 16 aa, synthetic construct
  REGION 1..16: note = synthetic
VRHGNFGTSYVSWFAY

SEQ ID NO: 95 - protein, 9 aa, synthetic construct
  REGION 1..9: note = synthetic
TGAVTTSNY

SEQ ID NO: 96-102 - skipped (7 entries)

SEQ ID NO: 103 - protein, 106 aa, synthetic construct
  REGION 1..106: note = synthetic
QIVLSQFPAIMSASPGEKVTMTCSASSSVSFMHWYQKKSGTSPKRWIYDTTKLASGVPARFTGSGSGTSYSLTISSMEAEDAATYYCQQWNSHPLTFGCGTKLELK

SEQ ID NO: 104 - protein, 113 aa, synthetic construct
  REGION 1..113: note = synthetic
QVQLQQPGAELVKPGTSVKLSCKASGYPFTNYWMHWVRDRPGQCLEWIGEINPSNGRTNYNEKFKSLATLTLDKSSSTAYMHLNSLTSEDSAVYYCARGFAYWGQGTLVTVSS

SEQ ID NO: 105 - protein, 113 aa, synthetic construct
  REGION 1..113: note = synthetic
QVQLQQPGAELVKPGTSVKLSCKASGYPFTNYWMHWVRQRPGQGLEWIGEINPSNGRTNYNEKFKSLATLTLDKSSSTAYMHLNSLTSEDSAVYYCARGFAYWGQGTLVTVSS

SEQ ID NO: 106 - protein, 109 aa, synthetic construct
  REGION 1..109: note = synthetic
QAVVTQEPSLTVSPGGTVTLTCRSSTGAVTTSNYANWVQKKPGQAPRGLIGGTNKRAPWTPARFSGSLLGGKAALTLSGAQAEDEADYYCALWYSNLWVFGGGTKLTVL

SEQ ID NO: 107 - protein, 125 aa, synthetic construct
  REGION 1..125: note = synthetic
EVQLVESGGGLVQPGGSLRLSCAASGFTFSTYAMNWVRDAPGKGLEWVGRIRSKYNNYATYYADSVKGRFTISRDDSKNSLYLQMNSLRAEDTAVYYCVRHGNFGNSYVSWFAYWGQGTLVTVSS

SEQ ID NO: 108 - protein, 125 aa, synthetic construct
  REGION 1..125: note = synthetic
EVQLVESGGGLVQPGGSLRLSCAASGFTFSTYAMNWVRQAPGKGLEWVGRIRSKYNNYATYYADSVKGRFTISRDDSKNSLYLQMNSLRAEDTAVYYCVRHGNFGNSYVSWFAYWGQGTLVTVSS

SEQ ID NO: 109 - protein, 107 aa, synthetic construct
  REGION 1..107: note = synthetic
DIQMTQSPSSLSASVGDRVTITCRASQDVNTAVAWYQDKPGKAPKLLIYSASFLYSGVPSRFSGSRSGTDFTLTISSLQPEDFATYYCQQAYTTPPTFGCGTKVEIK

SEQ ID NO: 110 - protein, 120 aa, synthetic construct
  REGION 1..120: note = synthetic
EVQLVESGGGLVQPGGSLRLSCAASGFNIKDTYIHWVRKAPGKCLEWVARIYPTNGYTRYADSVKGRFTISADTSKNTAYLQMNSLRAEDTAVYYCSRWGGDGFYAMDYWGQGTLVTVSS

SEQ ID NO: 111 - protein, 102 aa, synthetic construct
  REGION 1..102: note = synthetic
PSVDIFPPSDEQLKSGTASVVCLLNNFYPREAKVQWKVDNALQSGNSCESVTEQDSKDSTYSLSSTLTLSKADYEKHKVYACEVTHQGLSSPVTKSFNRGES

SEQ ID NO: 112 - protein, 103 aa, synthetic construct
  REGION 1..103: note = synthetic
ASTKGPSVFPLAPSSKSTSGGTAKLGCLVKDYFPEPVTVSWNSGALTSGVHTFPACLQSSGLYSLSSVVTVPSSSLGTQTYICNVNHKPSNTKVDKKVEPKSS